European Patent Specification EP 3 749 753 B1, published April 2, 2025. Title: METHODS FOR MANUFACTURING T CELLS. Applicant: Immatics Biotechnologies GmbH. The sequence listing filed with the application follows.

SEQUENCE LISTING (157 sequences)

SEQ ID NO: 1 - protein, 10 aa, Homo sapiens
YLYDSETKNA

SEQ ID NO: 2 - protein, 9 aa, Homo sapiens
HLMDQPLSV

SEQ ID NO: 3 - protein, 9 aa, Homo sapiens
GLLKKINSV

SEQ ID NO: 4 - protein, 9 aa, Homo sapiens
FLVDGSSAL

SEQ ID NO: 5 - protein, 10 aa, Homo sapiens
FLFDGSANLV

SEQ ID NO: 6 - protein, 9 aa, Homo sapiens
FLYKIIDEL

SEQ ID NO: 7 - protein, 11 aa, Homo sapiens
FILDSAETTTL

SEQ ID NO: 8 - protein, 9 aa, Homo sapiens
SVDVSPPKV

SEQ ID NO: 9 - protein, 8 aa, Homo sapiens
VADKIHSV

SEQ ID NO: 10 - protein, 9 aa, Homo sapiens
IVDDLTINL

SEQ ID NO: 11 - protein, 9 aa, Homo sapiens
GLLEELVTV

SEQ ID NO: 12 - protein, 10 aa, Homo sapiens
TLDGAAVNQV

SEQ ID NO: 13 - protein, 10 aa, Homo sapiens
SVLEKEIYSI

SEQ ID NO: 14 - protein, 9 aa, Homo sapiens
LLDPKTIFL

SEQ ID NO: 15 - protein, 9 aa, Homo sapiens
YTFSGDVQL

SEQ ID NO: 16 - protein, 9 aa, Homo sapiens
YLMDDFSSL

SEQ ID NO: 17 - protein, 9 aa, Homo sapiens
KVWSDVTPL

SEQ ID NO: 18 - protein, 11 aa, Homo sapiens
LLWGHPRVALA

SEQ ID NO: 19 - protein, 11 aa, Homo sapiens
KIWEELSVLEV

SEQ ID NO: 20 - protein, 9 aa, Homo sapiens
LLIPFTIFM

SEQ ID NO: 21 - protein, 9 aa, Homo sapiens
FLIENLLAA

SEQ ID NO: 22 - protein, 11 aa, Homo sapiens
LLWGHPRVALA

SEQ ID NO: 23 - protein, 9 aa, Homo sapiens
FLLEREQLL

SEQ ID NO: 24 - protein, 9 aa, Homo sapiens
SLAETIFIV

SEQ ID NO: 25 - protein, 9 aa, Homo sapiens
TLLEGISRA

SEQ ID NO: 26 - protein, 9 aa, Homo sapiens
ILQDGQFLV

SEQ ID NO: 27 - protein, 10 aa, Homo sapiens
VIFEGEPMYL

SEQ ID NO: 28 - protein, 9 aa, Homo sapiens
SLFESLEYL

SEQ ID NO: 29 - protein, 9 aa, Homo sapiens
SLLNQPKAV

SEQ ID NO: 30 - protein, 9 aa, Homo sapiens
GLAEFQENV

SEQ ID NO: 31 - protein, 9 aa, Homo sapiens
KLLAVIHEL

SEQ ID NO: 32 - protein, 9 aa, Homo sapiens
TLHDQVHLL

SEQ ID NO: 33 - protein, 11 aa, Homo sapiens
TLYNPERTITV

SEQ ID NO: 34 - protein, 9 aa, Homo sapiens
KLQEKIQEL

SEQ ID NO: 35 - protein, 10 aa, Homo sapiens
SVLEKEIYSI

SEQ ID NO: 36 - protein, 11 aa, Homo sapiens
RVIDDSLVVGV

SEQ ID NO: 37 - protein, 9 aa, Homo sapiens
VLFGELPAL

SEQ ID NO: 38 - protein, 9 aa, Homo sapiens
GLVDIMVHL

SEQ ID NO: 39 - protein, 9 aa, Homo sapiens
FLNAIETAL

SEQ ID NO: 40 - protein, 9 aa, Homo sapiens
ALLQALMEL

SEQ ID NO: 41 - protein, 9 aa, Homo sapiens
ALSSSQAEV

SEQ ID NO: 42 - protein, 11 aa, Homo sapiens
SLITGQDLLSV

SEQ ID NO: 43 - protein, 9 aa, Homo sapiens
QLIEKNWLL

SEQ ID NO: 44 - protein, 9 aa, Homo sapiens
LLDPKTIFL

SEQ ID NO: 45 - protein, 9 aa, Homo sapiens
RLHDENILL

SEQ ID NO: 46 - protein, 9 aa, Homo sapiens
YTFSGDVQL

SEQ ID NO: 47 - protein, 9 aa, Homo sapiens
GLPSATTTV

SEQ ID NO: 48 - protein, 11 aa, Homo sapiens
GLLPSAESIKL

SEQ ID NO: 49 - protein, 9 aa, Homo sapiens
KTASINQNV

SEQ ID NO: 50 - protein, 9 aa, Homo sapiens
SLLQHLIGL

SEQ ID NO: 51 - protein, 9 aa, Homo sapiens
YLMDDFSSL

SEQ ID NO: 52 - protein, 9 aa, Homo sapiens
LMYPYIYHV

SEQ ID NO: 53 - protein, 9 aa, Homo sapiens
KVWSDVTPL

SEQ ID NO: 54 - protein, 11 aa, Homo sapiens
LLWGHPRVALA

SEQ ID NO: 55 - protein, 9 aa, Homo sapiens
VLDGKVAVV

SEQ ID NO: 56 - protein, 9 aa, Homo sapiens
GLLGKVTSV

SEQ ID NO: 57 - protein, 9 aa, Homo sapiens
KMISAIPTL

SEQ ID NO: 58 - protein, 11 aa, Homo sapiens
GLLETTGLLAT

SEQ ID NO: 59 - protein, 9 aa, Homo sapiens
TLNTLDINL

SEQ ID NO: 60 - protein, 9 aa, Homo sapiens
VIIKGLEEI

SEQ ID NO: 61 - protein, 9 aa, Homo sapiens
YLEDGFAYV

SEQ ID NO: 62 - protein, 11 aa, Homo sapiens
KIWEELSVLEV

SEQ ID NO: 63 - protein, 9 aa, Homo sapiens
LLIPFTIFM

SEQ ID NO: 64 - protein, 10 aa, Homo sapiens
ISLDEVAVSL

SEQ ID NO: 65 - protein, 10 aa, Homo sapiens
KISDFGLATV

SEQ ID NO: 66 - protein, 11 aa, Homo sapiens
KLIGNIHGNEV

SEQ ID NO: 67 - protein, 9 aa, Homo sapiens
ILLSVLHQL

SEQ ID NO: 68 - protein, 9 aa, Homo sapiens
LDSEALLTL

SEQ ID NO: 69 - protein, 13 aa, Homo sapiens
VLQENSSDYQSNL

SEQ ID NO: 70 - protein, 11 aa, Homo sapiens
HLLGEGAFAQV

SEQ ID NO: 71 - protein, 9 aa, Homo sapiens
SLVENIHVL

SEQ ID NO: 72 - protein, 9 aa, Homo sapiens
YTFSGDVQL

SEQ ID NO: 73 - protein, 9 aa, Homo sapiens
SLSEKSPEV

SEQ ID NO: 74 - protein, 10 aa, Homo sapiens
AMFPDTIPRV

SEQ ID NO: 75 - protein, 9 aa, Homo sapiens
FLIENLLAA

SEQ ID NO: 76 - protein, 9 aa, Homo sapiens
FTAEFLEKV

SEQ ID NO: 77 - protein, 9 aa, Homo sapiens
ALYGNVQQV

SEQ ID NO: 78 - protein, 9 aa, Homo sapiens
LFQSRIAGV

SEQ ID NO: 79 - protein, 11 aa, Homo sapiens
ILAEEPIYIRV

SEQ ID NO: 80 - protein, 9 aa, Homo sapiens
FLLEREQLL

SEQ ID NO: 81 - protein, 10 aa, Homo sapiens
LLLPLELSLA

SEQ ID NO: 82 - protein, 9 aa, Homo sapiens
SLAETIFIV

SEQ ID NO: 83 - protein, 11 aa, Homo sapiens
AILNVDEKNQV

SEQ ID NO: 84 - protein, 9 aa, Homo sapiens
RLFEEVLGV

SEQ ID NO: 85 - protein, 9 aa, Homo sapiens
YLDEVAFML

SEQ ID NO: 86 - protein, 11 aa, Homo sapiens
KLIDEDEPLFL

SEQ ID NO: 87 - protein, 9 aa, Homo sapiens
KLFEKSTGL

SEQ ID NO: 88 - protein, 11 aa, Homo sapiens
SLLEVNEASSV

SEQ ID NO: 89 - protein, 10 aa, Homo sapiens
GVYDGREHTV

SEQ ID NO: 90 - protein, 10 aa, Homo sapiens
GLYPVTLVGV

SEQ ID NO: 91 - protein, 9 aa, Homo sapiens
ALLSSVAEA

SEQ ID NO: 92 - protein, 9 aa, Homo sapiens
TLLEGISRA

SEQ ID NO: 93 - protein, 9 aa, Homo sapiens
SLIEESEEL

SEQ ID NO: 94 - protein, 9 aa, Homo sapiens
ALYVQAPTV

SEQ ID NO: 95 - protein, 10 aa, Homo sapiens
KLIYKDLVSV

SEQ ID NO: 96 - protein, 9 aa, Homo sapiens
ILQDGQFLV

SEQ ID NO: 97 - protein, 9 aa, Homo sapiens
SLLDYEVSI

SEQ ID NO: 98 - protein, 9 aa, Homo sapiens
LLGDSSFFL

SEQ ID NO: 99 - protein, 10 aa, Homo sapiens
VIFEGEPMYL

SEQ ID NO: 100 - protein, 9 aa, Homo sapiens
ALSYILPYL

SEQ ID NO: 101 - protein, 9 aa, Homo sapiens
FLFVDPELV

SEQ ID NO: 102 - protein, 11 aa, Homo sapiens
SEWGSPHAAVP

SEQ ID NO: 103 - protein, 9 aa, Homo sapiens
ALSELERVL

SEQ ID NO: 104 - protein, 9 aa, Homo sapiens
SLFESLEYL

SEQ ID NO: 105 - protein, 9 aa, Homo sapiens
KVLEYVIKV

SEQ ID NO: 106 - protein, 10 aa, Homo sapiens
VLLNEILEQV

SEQ ID NO: 107 - protein, 9 aa, Homo sapiens
SLLNQPKAV

SEQ ID NO: 108 - protein, 9 aa, Homo sapiens
KMSELQTYV

SEQ ID NO: 109 - protein, 11 aa, Homo sapiens
ALLEQTGDMSL

SEQ ID NO: 110 - protein, 11 aa, Homo sapiens
VIIKGLEEITV

SEQ ID NO: 111 - protein, 9 aa, Homo sapiens
KQFEGTVEI

SEQ ID NO: 112 - protein, 9 aa, Homo sapiens
KLQEEIPVL

SEQ ID NO: 113 - protein, 9 aa, Homo sapiens
GLAEFQENV

SEQ ID NO: 114 - protein, 9 aa, Homo sapiens
NVAEIVIHI

SEQ ID NO: 115 - protein, 9 aa, Homo sapiens
ALAGIVTNV

SEQ ID NO: 116 - protein, 12 aa, Homo sapiens
NLLIDDKGTIKL

SEQ ID NO: 117 - protein, 10 aa, Homo sapiens
VLMQDSRLYL

SEQ ID NO: 118 - protein, 9 aa, Homo sapiens
KVLEHVVRV

SEQ ID NO: 119 - protein, 9 aa, Homo sapiens
LLWGNLPEI

SEQ ID NO: 120 - protein, 9 aa, Homo sapiens
SLMEKNQSL

SEQ ID NO: 121 - protein, 9 aa, Homo sapiens
KLLAVIHEL

SEQ ID NO: 122 - protein, 10 aa, Homo sapiens
ALGDKFLLRV

SEQ ID NO: 123 - protein, 11 aa, Homo sapiens
FLMKNSDLYGA

SEQ ID NO: 124 - protein, 10 aa, Homo sapiens
KLIDHQGLYL

SEQ ID NO: 125 - protein, 12 aa, Homo sapiens
GPGIFPPPPPQP

SEQ ID NO: 126 - protein, 9 aa, Homo sapiens
ALNESLVEC

SEQ ID NO: 127 - protein, 9 aa, Homo sapiens
GLAALAVHL

SEQ ID NO: 128 - protein, 9 aa, Homo sapiens
LLLEAVWHL

SEQ ID NO: 129 - protein, 9 aa, Homo sapiens
SIIEYLPTL

SEQ ID NO: 130 - protein, 9 aa, Homo sapiens
TLHDQVHLL

SEQ ID NO: 131 - protein, 9 aa, Homo sapiens
SLLMWITQC

SEQ ID NO: 132 - protein, 11 aa, Homo sapiens
FLLDKPQDLSI

SEQ ID NO: 133 - protein, 10 aa, Homo sapiens
YLLDMPLWYL

SEQ ID NO: 134 - protein, 9 aa, Homo sapiens
GLLDCPIFL

SEQ ID NO: 135 - protein, 9 aa, Homo sapiens
VLIEYNFSI

SEQ ID NO: 136 - protein, 11 aa, Homo sapiens
TLYNPERTITV

SEQ ID NO: 137 - protein, 9 aa, Homo sapiens
AVPPPPSSV

SEQ ID NO: 138 - protein, 9 aa, Homo sapiens
KLQEELNKV

SEQ ID NO: 139 - protein, 11 aa, Homo sapiens
KLMDPGSLPPL

SEQ ID NO: 140 - protein, 9 aa, Homo sapiens
ALIVSLPYL

SEQ ID NO: 141 - protein, 9 aa, Homo sapiens
FLLDGSANV

SEQ ID NO: 142 - protein, 10 aa, Homo sapiens
ALDPSGNQLI

SEQ ID NO: 143 - protein, 9 aa, Homo sapiens
ILIKHLVKV

SEQ ID NO: 144 - protein, 9 aa, Homo sapiens
VLLDTILQL

SEQ ID NO: 145 - protein, 9 aa, Homo sapiens
HLIAEIHTA

SEQ ID NO: 146 - protein, 9 aa, Homo sapiens
SMNGGVFAV

SEQ ID NO: 147 - protein, 9 aa, Homo sapiens
MLAEKLLQA

SEQ ID NO: 148 - protein, 9 aa, Homo sapiens
YMLDIFHEV

SEQ ID NO: 149 - protein, 11 aa, Homo sapiens
ALWLPTDSATV

SEQ ID NO: 150 - protein, 9 aa, Homo sapiens
GLASRILDA

SEQ ID NO: 151 - protein, 9 aa, Homo sapiens
SYVKVLHHL

SEQ ID NO: 152 - protein, 9 aa, Homo sapiens
VYLPKIPSW

SEQ ID NO: 153 - protein, 9 aa, Homo sapiens
NYEDHFPLL

SEQ ID NO: 154 - protein, 9 aa, Homo sapiens
VYIAELEKI

SEQ ID NO: 155 - protein, 12 aa, Homo sapiens
VHFEDTGKTLLF

SEQ ID NO: 156 - protein, 9 aa, Homo sapiens
VLSPFILTL

SEQ ID NO: 157 - protein, 9 aa, Homo sapiens
HLLEGSVGV